European Patent Application EP 4 582 545 A1, published July 9, 2025. Title: Monobody and NK cell. Applicant: GAIA BioMedicine Inc. The sequence listing filed with the application follows.

SEQUENCE LISTING (85 sequences)

SEQ ID NO: 1 - protein, 8 aa, synthetic construct
  REGION 1..8: note = part of monobody
PIWGRYGT

SEQ ID NO: 2 - protein, 10 aa, synthetic construct
  REGION 1..10: note = part of monobody
WTWLGYEYYW

SEQ ID NO: 3 - protein, 8 aa, synthetic construct
  REGION 1..8: note = part of monobody
TYWDWGFR

SEQ ID NO: 4 - protein, 12 aa, synthetic construct
  REGION 1..12: note = part of monobody
PGYYMWQRGVIN

SEQ ID NO: 5 - protein, 9 aa, synthetic construct
  REGION 1..9: note = part of monobody
RYKYHRRIN

SEQ ID NO: 6 - protein, 12 aa, synthetic construct
  REGION 1..12: note = part of monobody
GPIVSYSWWYHW

SEQ ID NO: 7 - protein, 10 aa, synthetic construct
  REGION 1..10: note = part of monobody
QAYWFEYTWW

SEQ ID NO: 8 - protein, 9 aa, synthetic construct
  REGION 1..9: note = part of monobody
TSPWVYNGY

SEQ ID NO: 9 - protein, 9 aa, synthetic construct
  REGION 1..9: note = part of monobody
TPPWIHKGW

SEQ ID NO: 10 - protein, 10 aa, synthetic construct
  REGION 1..10: note = part of monobody
LWHYYGDQYW

SEQ ID NO: 11 - protein, 12 aa, synthetic construct
  REGION 1..12: note = part of monobody
TDRNYDITYGMQ

SEQ ID NO: 12 - protein, 11 aa, synthetic construct
  REGION 1..11: note = part of monobody
WSWESYWHGTY

SEQ ID NO: 13 - protein, 12 aa, synthetic construct
  REGION 1..12: note = part of monobody
TVRGQTYYWWML

SEQ ID NO: 14 - protein, 10 aa, synthetic construct
  REGION 1..10: note = part of monobody
WDSKPGAIGI

SEQ ID NO: 15 - protein, 12 aa, synthetic construct
  REGION 1..12: note = part of monobody
WSWARRTHISWF

SEQ ID NO: 16 - protein, 12 aa, synthetic construct
  REGION 1..12: note = part of monobody
GQERAYGHPEHF

SEQ ID NO: 17 - protein, 16 aa, synthetic construct
  REGION 1..16: note = part of monobody
GTQWYVFNEAGDVAGY

SEQ ID NO: 18 - protein, 16 aa, synthetic construct
  REGION 1..16: note = part of monobody
VGYVNEKYDAWQSYVQ

SEQ ID NO: 19 - protein, 12 aa, synthetic construct
  REGION 1..12: note = part of monobody
LEWVYDDQWTSG

SEQ ID NO: 20 - protein, 12 aa, synthetic construct
  REGION 1..12: note = part of monobody
DQYKSWNLEEFH

SEQ ID NO: 21 - protein, 14 aa, synthetic construct
  REGION 1..14: note = part of monobody
VTPYGRKWVGMNGW

SEQ ID NO: 22 - protein, 12 aa, synthetic construct
  REGION 1..12: note = part of monobody
WMYVPEYYFNPW

SEQ ID NO: 23 - protein, 15 aa, synthetic construct
  REGION 1..15: note = part of monobody
YWWDGYSYSEEAWYY

SEQ ID NO: 24 - protein, 10 aa, synthetic construct
  REGION 1..10: note = part of monobody
TFMKDIPSYY

SEQ ID NO: 25 - protein, 13 aa, synthetic construct
  REGION 1..13: note = part of monobody
LEVVAPTSISWDA

SEQ ID NO: 26 - protein, 21 aa, synthetic construct
  REGION 1..21: note = part of monobody
MPNRLEVVEASPTSIQISWDA

SEQ ID NO: 27 - protein, 48 aa, synthetic construct
  REGION 1..48: note = part of monobody
VRYYRITYGETGGNSPVQEFTVPGSKSTATISGLKPGVDYTITVYAVT

SEQ ID NO: 28 - protein, 15 aa, synthetic construct
  REGION 1..15: note = part of monobody
PISINYRTEIDKPSQ

SEQ ID NO: 29 - protein, 29 aa, synthetic construct
  REGION 1..29: note = part of monobody
LEVVAPTSISWDAPAVTVRYYRITYGETG

SEQ ID NO: 30 - protein, 37 aa, synthetic construct
  REGION 1..37: note = part of monobody
  SITE 30: note = X can be any amino acid
  SITE 32: note = X can be any amino acid
MPNRLEVVEASPTSIQISWDAPAVTVRYYXIXYGETG

SEQ ID NO: 31 - protein, 32 aa, synthetic construct
  REGION 1..32: note = part of monobody
  SITE 3: note = X can be any amino acid
VQXFTVPGSKSTATISGLKPGVDYTITVYAVT

SEQ ID NO: 32 - protein, 104 aa, synthetic construct
  REGION 1..104: note = part of monobody
  SITE 26: note = X can be any amino acid
  SITE 28: note = X can be any amino acid
  SITE 48: note = X can be any amino acid
LEVVEASPTSIQISWDAPAVTVRYYXIXYGETGPGYYMWQRGVINVQXFTVPGSKSTATISGLKPGVDYTITVYAVTGQERAYGHPEHFPISINYRTEIDKPSQ

SEQ ID NO: 33 - protein, 105 aa, synthetic construct
  REGION 1..105: note = part of monobody
  SITE 26: note = X can be any amino acid
  SITE 28: note = X can be any amino acid
  SITE 45: note = X can be any amino acid
LEVVEASPTSIQISWDAPAVTVRYYXIXYGETGRYKYHRRINVQXFTVPGSKSTATISGLKPGVDYTITVYAVTGTQWYVFNEAGDVAGYPISINYRTEIDKPSQ

SEQ ID NO: 34 - protein, 101 aa, synthetic construct
  REGION 1..101: note = part of monobody
  SITE 26: note = X can be any amino acid
  SITE 28: note = X can be any amino acid
  SITE 45: note = X can be any amino acid
LEVVEASPTSIQISWDAPAVTVRYYXIXYGETGTSPWVYNGYVQXFTVPGSKSTATISGLKPGVDYTITVYAVTDQYKSWNLEEFHPISINYRTEIDKPSQ

SEQ ID NO: 35 - protein, 103 aa, synthetic construct
  REGION 1..103: note = part of monobody
  SITE 26: note = X can be any amino acid
  SITE 28: note = X can be any amino acid
  SITE 45: note = X can be any amino acid
LEVVEASPTSIQISWDAPAVTVRYYXIXYGETGTPPWIHKGWVQXFTVPGSKSTATISGLKPGVDYTITVYAVTVTPYGRKWVGMNGWPISINYRTEIDKPSQ

SEQ ID NO: 36 - protein, 101 aa, synthetic construct
  REGION 1..101: note = part of monobody
  SITE 26: note = X can be any amino acid
  SITE 28: note = X can be any amino acid
  SITE 47: note = X can be any amino acid
LEVVEASPTSIQISWDAPAVTVRYYXIXYGETGWSWESYWHGTYVQXFTVPGSKSTATISGLKPGVDYTITVYAVTTFMKDIPSYYPISINYRTEIDKPSQ

SEQ ID NO: 37 - protein, 104 aa, synthetic construct
  REGION 1..104: note = part of monobody
LEVVEASPTSIQISWDAPAVTVRYYDIYYGETGPGYYMWQRGVINVQAFTVPGSKSTATISGLKPGVDYTITVYAVTGQERAYGHPEHFPISINYRTEIDKPSQ

SEQ ID NO: 38 - protein, 105 aa, synthetic construct
  REGION 1..105: note = part of monobody
LEVVEASPTSIQISWDAPAVTVRYYVISYGETGRYKYHRRINVQGFTVPGSKSTATISGLKPGVDYTITVYAVTGTQWYVFNEAGDVAGYPISINYRTEIDKPSQ

SEQ ID NO: 39 - protein, 101 aa, synthetic construct
  REGION 1..101: note = part of monobody
LEVVEASPTSIQISWDAPAVTVRYYGIYYGETGTSPWVYNGYVQEFTVPGSKSTATISGLKPGVDYTITVYAVTDQYKSWNLEEFHPISINYRTEIDKPSQ

SEQ ID NO: 40 - protein, 103 aa, synthetic construct
  REGION 1..103: note = part of monobody
LEVVEASPTSIQISWDAPAVTVRYYEILYGETGTPPWIHKGWVQYFTVPGSKSTATISGLKPGVDYTITVYAVTVTPYGRKWVGMNGWPISINYRTEIDKPSQ

SEQ ID NO: 41 - protein, 101 aa, synthetic construct
  REGION 1..101: note = part of monobody
LEVVEASPTSIQISWDAPAVTVRYYVITYGETGWSWESYWHGTYVQQFTVPGSKSTATISGLKPGVDYTITVYAVTTFMKDIPSYYPISINYRTEIDKPSQ

SEQ ID NO: 42 - protein, 100 aa, synthetic construct
  REGION 1..100: note = part of monobody
LEVVEASPTSIQISWDAPIWGRYGTVRYYRITYGETGGNSPVQEFTVPGSKSTATISGLKPGVDYTITVYAVTTVRGQTYYWWMLPISINYRTEIDKPSQ

SEQ ID NO: 43 - protein, 100 aa, synthetic construct
  REGION 1..100: note = part of monobody
LEVVEASPTSIQISWDAWTWLGYEYYWVRYYRITYGETGGNSPVQEFTVPGSKSTATISGLKPGVDYTITVYAVTWDSKPGAIGIPISINYRTEIDKPSQ

SEQ ID NO: 44 - protein, 100 aa, synthetic construct
  REGION 1..100: note = part of monobody
LEVVEASPTSIQISWDATYWDWGFRVRYYRITYGETGGNSPVQEFTVPGSKSTATISGLKPGVDYTITVYAVTWSWARRTHISWFPISINYRTEIDKPSQ

SEQ ID NO: 45 - protein, 108 aa, synthetic construct
  REGION 1..108: note = part of monobody
LEVVEASPTSIQISWDAGPIVSYSWWYHWVRYYRITYGETGGNSPVQEFTVPGSKSTATISGLKPGVDYTITVYAVTVGYVNEKYDAWQSYVQPISINYRTEIDKPSQ

SEQ ID NO: 46 - protein, 102 aa, synthetic construct
  REGION 1..102: note = part of monobody
LEVVEASPTSIQISWDAQAYWFEYTWWVRYYRITYGETGGNSPVQEFTVPGSKSTATISGLKPGVDYTITVYAVTLEWVYDDQWTSGPISINYRTEIDKPSQ

SEQ ID NO: 47 - protein, 102 aa, synthetic construct
  REGION 1..102: note = part of monobody
LEVVEASPTSIQISWDALWHYYGDQYWVRYYRITYGETGGNSPVQEFTVPGSKSTATISGLKPGVDYTITVYAVTWMYVPEYYFNPWPISINYRTEIDKPSQ

SEQ ID NO: 48 - protein, 107 aa, synthetic construct
  REGION 1..107: note = part of monobody
LEVVEASPTSIQISWDATDRNYDITYGMQVRYYRITYGETGGNSPVQEFTVPGSKSTATISGLKPGVDYTITVYAVTYWWDGYSYSEEAWYYPISINYRTEIDKPSQ

SEQ ID NO: 49 - DNA, 405 bp, synthetic construct
  misc_feature 1..405: note = mRNA of BC-FG library
  misc_feature 84..85: note = n is a, c, g, or t
  misc_feature 87..88: note = n is a, c, g, or t
  misc_feature 90..91: note = n is a, c, g, or t
  misc_feature 93..94: note = n is a, c, g, or t
  misc_feature 96..97: note = n is a, c, g, or t
  misc_feature 99..100: note = n is a, c, g, or t
  misc_feature 102..103: note = n is a, c, g, or t
  misc_feature 105..106: note = n is a, c, g, or t
  misc_feature 108..109: note = n is a, c, g, or t
  misc_feature 111..112: note = n is a, c, g, or t
  misc_feature 114..115: note = n is a, c, g, or t
  misc_feature 117..118: note = n is a, c, g, or t
  misc_feature 264..265: note = n is a, c, g, or t
  misc_feature 267..268: note = n is a, c, g, or t
  misc_feature 270..271: note = n is a, c, g, or t
  misc_feature 273..274: note = n is a, c, g, or t
  misc_feature 276..277: note = n is a, c, g, or t
  misc_feature 279..280: note = n is a, c, g, or t
  misc_feature 282..283: note = n is a, c, g, or t
  misc_feature 285..286: note = n is a, c, g, or t
  misc_feature 288..289: note = n is a, c, g, or t
  misc_feature 291..292: note = n is a, c, g, or t
  misc_feature 294..295: note = n is a, c, g, or t
  misc_feature 297..298: note = n is a, c, g, or t
  misc_feature 300..301: note = n is a, c, g, or t
  misc_feature 303..304: note = n is a, c, g, or t
  misc_feature 306..307: note = n is a, c, g, or t
  misc_feature 309..310: note = n is a, c, g, or t
  misc_feature 312..313: note = n is a, c, g, or t
  misc_feature 315..316: note = n is a, c, g, or t
  source 1..405: mol_type = other DNA
  misc_feature 102..119: note = One or more (NNK) in this region may be deleted
  misc_feature 294..317: note = One or more [NNK] in this region may be deleted
ggattaaggaggtgatatttatgcctaatcgtctagaagttgttgaagcgtcccccaccagcattcagatcagctgggatgctnnknnknnknnknnknnknnknnknnknnknnknnkgtgcgttattaccgtatcacttacggagaaacaggaggaaatagccctgtccaggagttcactgtgcctgggagcaagtctacagctaccatcagcggccttaaacctggagttgattataccatcactgtgtatgctgtcactnnknnknnknnknnknnknnknnknnknnknnknnknnknnknnknnknnknnkccaatttccattaattaccgtacagaaattgacaaaccaagtcaaggtggaggaggaggccgatagtggacggcgggcgcgaggcggg

SEQ ID NO: 50 - protein, 120 aa, synthetic construct
  REGION 1..120: note = BC-FG library
  REGION 22..33: note = X can be any amino acid
  REGION 82..99: note = X can be any amino acid
  REGION 28..33: note = One or more X in this region may be deleted
  REGION 92..99: note = One or more X in this region may be deleted
MPNRLEVVEASPTSIQISWDAXXXXXXXXXXXXVRYYRITYGETGGNSPVQEFTVPGSKSTATISGLKPGVDYTITVYAVTXXXXXXXXXXXXXXXXXXPISINYRTEIDKPSQGGGGGR

SEQ ID NO: 51 - DNA, 402 bp, synthetic construct
  misc_feature 1..402: note = mRNA of CD-FG library
  misc_feature 108..109: note = n is a, c, g, or t
  misc_feature 114..115: note = n is a, c, g, or t
  misc_feature 132..133: note = n is a, c, g, or t
  misc_feature 135..136: note = n is a, c, g, or t
  misc_feature 138..139: note = n is a, c, g, or t
  misc_feature 141..142: note = n is a, c, g, or t
  misc_feature 144..145: note = n is a, c, g, or t
  misc_feature 147..148: note = n is a, c, g, or t
  misc_feature 150..151: note = n is a, c, g, or t
  misc_feature 153..154: note = n is a, c, g, or t
  misc_feature 156..157: note = n is a, c, g, or t
  misc_feature 159..160: note = n is a, c, g, or t
  misc_feature 162..163: note = n is a, c, g, or t
  misc_feature 171..172: note = n is a, c, g, or t
  misc_feature 261..262: note = n is a, c, g, or t
  misc_feature 264..265: note = n is a, c, g, or t
  misc_feature 267..268: note = n is a, c, g, or t
  misc_feature 270..271: note = n is a, c, g, or t
  misc_feature 273..274: note = n is a, c, g, or t
  misc_feature 276..277: note = n is a, c, g, or t
  misc_feature 279..280: note = n is a, c, g, or t
  misc_feature 282..283: note = n is a, c, g, or t
  misc_feature 285..286: note = n is a, c, g, or t
  misc_feature 288..289: note = n is a, c, g, or t
  misc_feature 291..292: note = n is a, c, g, or t
  misc_feature 294..295: note = n is a, c, g, or t
  misc_feature 297..298: note = n is a, c, g, or t
  misc_feature 300..301: note = n is a, c, g, or t
  misc_feature 303..304: note = n is a, c, g, or t
  misc_feature 306..307: note = n is a, c, g, or t
  misc_feature 309..310: note = n is a, c, g, or t
  misc_feature 312..313: note = n is a, c, g, or t
  source 1..402: mol_type = other DNA
  misc_feature 159..164: note = One or more [NNK] in this region may be deleted
  misc_feature 290..314: note = One or more [NNK] in this region may be deleted
ggattaaggaggtgatatttatgcctaatcgtctagaagttgttgaagcgtcccccaccagcattcagatcagctgggatgctcctgctgtcacagtgcgttattacnnkatcnnktacggagaaacaggannknnknnknnknnknnknnknnknnknnknnkgtccagnnkttcactgtgcctgggagcaagtctacagctaccatcagcggccttaaacctggagttgattataccatcactgtgtatgctgtcactnnknnknnknnknnknnknnknnknnknnknnknnknnknnknnknnknnknnkccaatttccattaattaccgtacagaaattgacaaaccaagtcaaggtggaggaggaggccgatagtggacggcgggcgcgaggcggg

SEQ ID NO: 52 - protein, 119 aa, synthetic construct
  REGION 1..119: note = BC-FG library
  SITE 30: note = X can be any amino acid
  SITE 32: note = X can be any amino acid
  REGION 38..48: note = X can be any amino acid
  SITE 51: note = X can be any amino acid
  REGION 81..98: note = X can be any amino acid
  REGION 47..48: note = One or more X in this region may be deleted
  REGION 91..98: note = One or more X in this region may be deleted
MPNRLEVVEASPTSIQISWDAPAVTVRYYXIXYGETGXXXXXXXXXXXVQXFTVPGSKSTATISGLKPGVDYTITVYAVTXXXXXXXXXXXXXXXXXXPISINYRTEIDKPSQGGGGGR

SEQ ID NO: 53 - DNA, 44 bp, synthetic construct
  misc_feature 1..44: note = T7SD8M2.F44
  source 1..44: mol_type = other DNA
atactaatacgactcactataggattaaggaggtgatatttatg

SEQ ID NO: 54 - DNA, 20 bp, synthetic construct
  misc_feature 1..20: note = MoS-RealTime.R20
  source 1..20: mol_type = other DNA
agcatcccagctgatctgaa

SEQ ID NO: 55 - DNA, 28 bp, synthetic construct
  misc_feature 1..28: note = Mos G5R-T.R28
  source 1..28: mol_type = other DNA
actatcggcctcctcctccaccttgact

SEQ ID NO: 56 - DNA, 47 bp, synthetic construct
  misc_feature 1..47: note = T7SD8M2P.F47
  source 1..47: mol_type = other DNA
atactaatacgactcactataggattaaggaggtgatatttatgcct

SEQ ID NO: 57 - DNA, 45 bp, synthetic construct
  misc_feature 1..45: note = Mos-G5R-T-an21-3.R45
  source 1..45: mol_type = other DNA
cccgcctcgcgcccgccgtccactatcggcctcctcctccacctt

SEQ ID NO: 58 - DNA, 40 bp, synthetic construct
  misc_feature 1..40: note = Mb-NKp46- BC-1 F40
  source 1..40: mol_type = other DNA
ttcagatcagctgggatgctccgatctggggtcgttacgg

SEQ ID NO: 59 - DNA, 40 bp, synthetic construct
  misc_feature 1..40: note = Mb-NKp46- BC-2 F40
  source 1..40: mol_type = other DNA
ttcagatcagctgggatgcttggacttggctcggttacga

SEQ ID NO: 60 - DNA, 44 bp, synthetic construct
  misc_feature 1..44: note = Mb-NKp46- BC-3 F44
  source 1..44: mol_type = other DNA
ttcagatcagctgggatgctacttactgggactggggtttccgt

SEQ ID NO: 61 - DNA, 40 bp, synthetic construct
  misc_feature 1..40: note = Mb-2B4-BC-1 F40
  source 1..40: mol_type = other DNA
ttcagatcagctgggatgctggtccgatcgtttcttactc

SEQ ID NO: 62 - DNA, 40 bp, synthetic construct
  misc_feature 1..40: note = Mb-2B4-BC-2 F40
  source 1..40: mol_type = other DNA
ttcagatcagctgggatgctcaggcttactggttcgaata

SEQ ID NO: 63 - DNA, 40 bp, synthetic construct
  misc_feature 1..40: note = Mb-NKp30- BC-2 F40
  source 1..40: mol_type = other DNA
ttcagatcagctgggatgctctgtggcattactacggtga

SEQ ID NO: 64 - DNA, 40 bp, synthetic construct
  misc_feature 1..40: note = Mb-NKp30- BC-6 F40
  source 1..40: mol_type = other DNA
ttcagatcagctgggatgctactgaccgtaactacgacat

SEQ ID NO: 65 - DNA, 65 bp, synthetic construct
  misc_feature 1..65: note = Mb-NKp46- CD-1 F65
  source 1..65: mol_type = other DNA
gctgtcacagtgcgttattacgacatctactacggagaaacaggaccgggttactacatgtggca

SEQ ID NO: 66 - DNA, 65 bp, synthetic construct
  misc_feature 1..65: note = Mb-NKp46- CD-3 F65
  source 1..65: mol_type = other DNA
gctgtcacagtgcgttattacgttatctcttacggagaaacaggacgttacaaataccatcgtcg

SEQ ID NO: 67 - DNA, 65 bp, synthetic construct
  misc_feature 1..65: note = Mb-2B4-CD-1 F65
  source 1..65: mol_type = other DNA
gctgtcacagtgcgttattacggtatctactacggagaaacaggaacttctccgtgggtttacaa

SEQ ID NO: 68 - DNA, 65 bp, synthetic construct
  misc_feature 1..65: note = Mb-2B4-CD-3 F65
  source 1..65: mol_type = other DNA
gctgtcacagtgcgttattacgaaatcctgtacggagaaacaggaactccgccgtggatccataa

SEQ ID NO: 69 - DNA, 78 bp, synthetic construct
  misc_feature 1..78: note = Mb-NKp30- CD-9 F78
  source 1..78: mol_type = other DNA
gctgtcacagtgcgttattacgttatcacttacggagaaacaggatggtcttgggaatcttactggcatggtacttac

SEQ ID NO: 70 - DNA, 40 bp, synthetic construct
  misc_feature 1..40: note = Mb-NKp46- BC-1 R40
  source 1..40: mol_type = other DNA
cggtaattaatggaaattggcagcatccaccagtagtaag

SEQ ID NO: 71 - DNA, 40 bp, synthetic construct
  misc_feature 1..40: note = Mb-NKp46- BC-2 R40
  source 1..40: mol_type = other DNA
cggtaattaatggaaattgggataccgatagcacccggtt

SEQ ID NO: 72 - DNA, 40 bp, synthetic construct
  misc_feature 1..40: note = Mb-NKp46- BC-3 R40
  source 1..40: mol_type = other DNA
cggtaattaatggaaattgggaaccaagagatatgagtac

SEQ ID NO: 73 - DNA, 40 bp, synthetic construct
  misc_feature 1..40: note = Mb-2B4-BC-1 R40
  source 1..40: mol_type = other DNA
cggtaattaatggaaattggctgaacgtaagactgccaag

SEQ ID NO: 74 - DNA, 40 bp, synthetic construct
  misc_feature 1..40: note = Mb-2B4-BC-2 R40
  source 1..40: mol_type = other DNA
cggtaattaatggaaattggaccagaagtccactggtcgt

SEQ ID NO: 75 - DNA, 40 bp, synthetic construct
  misc_feature 1..40: note = Mb-NKp30- BC-2 R40
  source 1..40: mol_type = other DNA
cggtaattaatggaaattggccacgggttgaagtagtatt

SEQ ID NO: 76 - DNA, 41 bp, synthetic construct
  misc_feature 1..41: note = Mb-NKp30- BC-6 R41
  source 1..41: mol_type = other DNA
cggtaattaatggaaattgggtagtaccaagcttcttcaga

SEQ ID NO: 77 - DNA, 40 bp, synthetic construct
  misc_feature 1..40: note = Mb-NKp46- CD-1 R40
  source 1..40: mol_type = other DNA
cggtaattaatggaaattgggaaatgttccggatgaccgt

SEQ ID NO: 78 - DNA, 40 bp, synthetic construct
  misc_feature 1..40: note = Mb-NKp46- CD-3 R40
  source 1..40: mol_type = other DNA
cggtaattaatggaaattgggtaaccagcaacgtcaccag

SEQ ID NO: 79 - DNA, 40 bp, synthetic construct
  misc_feature 1..40: note = Mb-2B4-CD-1 R40
  source 1..40: mol_type = other DNA
cggtaattaatggaaattggatggaattcttccaggttcc

SEQ ID NO: 80 - DNA, 40 bp, synthetic construct
  misc_feature 1..40: note = Mb-2B4-CD-3 R40
  source 1..40: mol_type = other DNA
cggtaattaatggaaattggccaaccgttcataccaaccc

SEQ ID NO: 81 - DNA, 50 bp, synthetic construct
  misc_feature 1..50: note = Mb-NKp30- CD-9 R50
  source 1..50: mol_type = other DNA
cggtaattaatggaaattgggtagtaagacgggatgtctttcatgaaagt

SEQ ID NO: 82 - protein, 90 aa, Homo sapiens
LEVVAPTSISWDAPAVTVRYYRITYGETGGNSPVQEFTVPGSKSTATISGLKPGVDYTITVYAVTGRGDSPASSKPISINYRTEIDKPSQ

SEQ ID NO: 83 - protein, 4 aa, synthetic construct
PAVT

SEQ ID NO: 84 - protein, 4 aa, synthetic construct
GNSP

SEQ ID NO: 85 - protein, 10 aa, synthetic construct
GRGDSPASSK